European Patent Application EP 4 458 955 A1, published November 6, 2024. Title: Factor for direct Conversion into motor neuron. Applicant: 주식회사 스탠드업테라퓨티스. The sequence listing filed with the application follows.

SEQUENCE LISTING (36 sequences)

SEQ ID NO: 1 - protein, 222 aa, synthetic construct
MAARPKLHYPNGRGRMESVRWVLAAAGVEFDEEFLETKEQLYKLQDGNHLLFQQVPMVEIDGMKLVQTRSILHYIADKHNLFGKNLKERTLIDMYVEGTLDLLELLIMHPFLKPDDQQKEVVNMAQKAIIRYFPVFEKILRGHGQSFLVGNQLSLADVILLQTILALEEKIPNILSAFPFLQEYTVKLSNIPTIKRFLEPGSKKKPPPDEIYVRTVYNIFRP

SEQ ID NO: 2 - DNA, 1240 bp, synthetic construct
  source 1..1240: mol_type = other DNA
gctttgtgcggctccaggcctccgagtggactccagaaagcctgaaaagctatcatggcagcaaggcccaagctccactatcccaacggaagaggccggatggagtccgtgagatgggttttagctgccgccggagtcgagtttgatgaagaatttctggaaacaaaagaacagttgtacaagttgcaggatggtaaccacctgctgttccaacaagtgcccatggttgaaattgacgggatgaagttggtacagacccgaagcattctccactacatagcagacaagcacaatctctttggcaagaacctcaaggagagaaccctgattgacatgtacgtggaggggacactggatctgctggaactgcttatcatgcatcctttcttaaaaccagatgatcagcaaaaggaagtggttaacatggcccagaaggctataattagatactttcctgtgtttgaaaagattttaaggggtcacggacaaagctttcttgttggtaatcagctgagccttgcagatgtgattttactccaaaccattttagctctagaagagaaaattcctaatatcctgtctgcatttcctttcctccaggaatacacagtgaaactaagtaatatccctacaattaagagattccttgaacctggcagcaagaagaagcctccccctgatgaaatttatgtgagaaccgtctacaacatctttaggccataaaacaacacatccatgtgtgagtgacagtgtgttcctagagatggtattgtctacagtcatgtcttaatggatcccagctctgtcatggtgctatctatgtattaagttgggtcctaagttgggtcttttgtgtcaacgagatcatctcttctagaaatatcaaccttttttgtccagtaaataattgttaggggatctttattggaaaacttttttggagaggctggtatttaagttagatctgattgggctactcatgtcctgtagccagttcatcctcataataagaatgggcaggatctcttgttctctcctgagtgtctttctactctcctgagcgtctttctgctctccttatcctgttctcttatccttatcccctccagtctctgcctaatttttagtgtttaataacaaccgaatgtctagtaaatgactctcctctgagctgtaataaataaaatggtagtaatgaatgcaatcagtattagccaaaataaagaatttatgagtcatt

SEQ ID NO: 3 - DNA, 9536 bp, synthetic construct
  source 1..9536: mol_type = other DNA
cgccatgttgacattgattattgactagttattaatagtaatcaattacggggtcattagttcatagcccatatatggagttccgcgttacataacttacggtaaatggcccgcctggctgaccgcccaacgacccccgcccattgacgtcaataatgacgtatgttcccatagtaacgccaatagggactttccattgacgtcaatgggtggagtatttacggtaaactgcccacttggcagtacatcaagtgtatcatatgccaagtacgccccctattgacgtcaatgacggtaaatggcccgcctggcattatgcccagtacatgaccttatgggactttcctacttggcagtacatctacgtattagtcatcgctattaccatggtgatgcggttttggcagtacatcaatgggcgtggatagcggtttgactcacggggatttccaagtctccaccccattgacgtcaatgggagtttgttttggcaccaaaatcaacgggactttccaaaatgtcgtaacaactccgccccattgacgcaaatgggcggtaggcgtgtacggtgggaggtctatataagcagagctcgtttagtgaaccgtcagatcgcctggagacgccatccacgctgttttgacctccatagaagacaccgggaccgatccagcctcccctcgaagcttacatgtggtaccatggaaagctctgccaagatggagagcggcggcgccggccagcagccccagccgcagccccagcagcccttcctgccgcccgcagcctgtttctttgccacggccgcagccgcggcggccgcagccgccgcagcggcagcgcagagcgcgcagcagcagcagcagcagcagcagcagcagcagcaggcgccgcagctgagaccggcggccgacggccagccctcagggggcggtcacaagtcagcgcccaagcaagtcaagcgacagcgctcgtcttcgcccgaactgatgcgctgcaaacgccggctcaacttcagcggctttggctacagcctgccgcagcagcagccggccgccgtggcgcgccgcaacgagcgcgagcgcaaccgcgtcaagttggtcaacctgggctttgccacccttcgggagcacgtccccaacggcgcggccaacaagaagatgagtaaggtggagacactgcgctcggcggtcgagtacatccgcgcgctgcagcagctgctggacgagcatgacgcggtgagcgccgccttccaggcaggcgtcctgtcgcccaccatctcccccaactactccaacgacttgaactccatggccggctcgccggtctcatcctactcgtcggacgagggctcttacgacccgctcagccccgaggagcaggagcttctcgacttcaccaactggttcggcagtggagagggcagaggaagtctgctaacatgcggtgacgtcgaggagaatcctggcccaatgttcgtcaaatccgagaccttggagttgaaggaggaagaggacgtgttagtgctgctcggatcggcctcccccgccttggcggccctgaccccgctgtcatccagcgccgacgaagaagaggaggaggagccgggcgcgtcaggcggggcgcgtcggcagcgcggggctgaggccgggcagggggcgcggggcggcgtggctgcgggtgcggagggctgccggcccgcacggctgctgggtctggtacacgattgcaaacggcgcccttcccgggcgcgggccgtctcccgaggcgccaagacggccgagacggtgcagcgcatcaagaagacccgtagactgaaggccaacaaccgcgagcgaaaccgcatgcacaacctcaacgcggcactggacgcgctgcgcgaggtgctccccacgttccccgaggacgccaagctcaccaagatcgagaccctgcgcttcgcccacaactacatctgggcactcaccgagaccctgcgcctggcggatcactgcgggggcggcggcgggggcctgccgggggcgctcttctccgaggcagtgttgctgagcccgggaggcgccagcgccgccctgagcagcagcggagacagcccctcgcccgcctccacgtggagttgcaccaacagccccgcgccgtcctcctccgtgtcctccaattccacctccccctacagctgcactttatcgcccgccagcccggccgggtcagacatggactattggcagcccccacctcccgacaagcaccgctatgcacctcacctccccatagccagggattgtatcttgggatccggagctactaacttcagcctgctgaagcaggctggagacgtggaggagaaccctggacctatgggagacatgggagatccaccaaaaaaaaaacgtctgatttccctatgtgttggttgcggcaatcagattcacgatcagtatattctgagggtttctccggatttggaatggcatgcggcatgtttgaaatgtgcggagtgtaatcagtatttggacgagagctgtacatgctttgttagggatgggaaaacctactgtaaaagagattatatcaggttgtacgggatcaaatgcgccaagtgcagcatcggcttcagcaagaacgacttcgtgatgcgtgcccgctccaaggtgtatcacatcgagtgtttccgctgtgtggcctgcagccgccagctcatccctggggacgaatttgcgcttcgggaggacggtctcttctgccgagcagaccacgatgtggtggagagggccagtctaggcgctggcgacccgctcagtcccctgcatccagcgcggccactgcaaatggcagcggagcccatctccgccaggcagccggccctgcggccccacgtccacaagcagccggagaagaccacccgcgtgcggactgtgctgaacgagaagcagctgcacaccttgcggacctgctacgccgcaaacccgcggccagatgcgctcatgaaggagcaactggtagagatgacgggcctcagtccccgtgtgatccgggtctggtttcaaaacaagcggtgcaaggacaagaagcgaagcatcatgatgaagcaactccagcagcagcagcccaatgacaaaactaatatccaggggatgacaggaactcccatggtggctgccagtccagagagacacgacggtggcttacaggctaacccagtggaagtacaaagttaccagccaccttggaaagtactgagcgacttcgccttgcagagtgacatagatcagcctgcttttcagcaactggtcaatttttcagaaggaggaccgggctctaattccactggcagtgaagtagcatcaatgtcctctcaacttccagatacacctaacagcatggtagccagtcctattgaggcattgatgcacagcagaggctctggcgagggcagaggcagcctgctgacatgtggcgacgtggaagagaaccctggccccggtaccatggaagccagaggcgaactgggccctgccagagaatctgccggcggagatctgctgctggccctgctggctagaagggccgacctgagaagagaaatccccctgtgcgccggctgcgaccagcacatcctggaccggtttatcctgaaggccctggacagacactggcacagcaagtgcctgaagtgcagcgactgccacacccccctggccgagagatgctttagcagaggcgagagcgtgtactgcaaggacgacttcttcaagagattcggcaccaagtgcgccgcctgccagctgggaattcctcctacacaggtcgtgcggagagcccaggacttcgtgtaccatctgcactgcttcgcctgcgtcgtgtgcaagagacagctggccaccggcgacgagttctacctgatggaagatagccggctcgtgtgtaaagccgactacgagacagccaagcagagagaggccgaggccaccgccaaaagacccagaaccaccatcaccgccaagcagctggaaaccctgaagtccgcctacaacaccagccccaagcccgccagacatgtgcgggaacagctgagcagcgagacaggcctggacatgagagtggtgcaagtgtggttccagaacagacgggccaaagagaagcggctgaagaaggacgccggcaggcagagatggggccagtacttccggaacatgaagcggtccagaggcggcagcaagagcgacaaggacagcgtgcaggaaggccaggacagcgacgccgaggtgtccttcccagatgagcctagcctggccgaaatgggcccagccaatggcctgtatggcagcctgggagagccaacccaggctctgggcagaccttctggcgccctgggcaacttctctctggaacacggcggactggccggacccgagcagtatagagaactgaggcccggcagcccttacggcgtgccaccttctccagctgcccctcagtctctgccaggacctcagcctctgctgtccagcctggtgtaccccgatacaagcctgggcctggtgccatctggcgctccaggcggacctcctccaatgagagtgctggccggcaatggccctagcagcgatctgagcacaggcagctctggcggctaccccgattttcctgccagccctgcctcctggctggacgaagtggatcacgcccagttctgagcggccgctctagaggatccaagcttatcgataccgtcgacctcgagggcccagatctaattcaccccaccagtgcaggctgcctatcagaaagtggtggctggtgtggctaatgccctggcccacaagtatcactaagctcgctttcttgctgtccaatttctattaaaggttcctttgttccctaagtccaactactaaactgggggatattatgaagggccttgagcatctggattctgcctaataaaaaacatttattttcattgcaatgatgtatttaaattatttctgaatattttactaaaaagggaatgtgggaggtcagtgcatttaaaacataaagaaatgaagagctagttcaaaccttgggaaaatacactatatcttaaactccatgaaagaaggtgaggctgcaaacagctaatgcacattggcaacagcccctgatgcctatgccttattcatccctcagaaaaggattcaagtagaggcttgatttggaggttaaagttttgctatgctgtattttacattacttattgttttagctgtcctcatgaatgtcttttcactacccatttgcttatcctgcatctctcagccttgactccactcagttctcttgcttagagataccacctttcccctgaagtgttccttccatgttttacggcgagatggtttctcctcgcctggccactcagccttagttgtctctgttgtcttatagaggtctacttgaagaaggaaaaacagggggcatggtttgactgtcctgtgagcccttcttccctgcctcccccactcacagtgacccggaatccctcgacatctagagcatggctacgtagataagtagcatggcgggttaatcattaactacaaggaacccctagtgatggagttggccactccctctctgcgcgctcgctcgctcactgaggccgggcgaccaaaggtcgcccgacgcccgggctttgcccgggcggcctcagtgagcgagcgagcgcgcagctggcgtaatagcgaagaggcccgcaccgatcgcccttcccaacagttgcgcagcctgaatggcgaatggcgattccgttgcaatggctggcggtaatattgttctggatattaccagcaaggccgatagtttgagttcttctactcaggcaagtgatgttattactaatcaaagaagtattgcgacaacggttaatttgcgtgatggacagactcttttactcggtggcctcactgattataaaaacacttctcaggattctggcgtaccgttcctgtctaaaatccctttaatcggcctcctgtttagctcccgctctgattctaacgaggaaagcacgttatacgtgctcgtcaaagcaaccatagtacgcgccctgtagcggcgcattaagcgcggcgggtgtggtggttacgcgcagcgtgaccgctacacttgccagcgccctagcgcccgctcctttcgctttcttcccttcctttctcgccacgttcgccggctttccccgtcaagctctaaatcgggggctccctttagggttccgatttagtgctttacggcacctcgaccccaaaaaacttgattagggtgatggttcacgtagtgggccatcgccctgatagacggtttttcgccctttgacgttggagtccacgttctttaatagtggactcttgttccaaactggaacaacactcaaccctatctcggtctattcttttgatttataagggattttgccgatttcggcctattggttaaaaaatgagctgatttaacaaaaatttaacgcgaattttaacaaaatattaacgcttacaatttaaatatttgcttatacaatcttcctgtttttggggcttttctgattatcaaccggggtacatatgattgacatgctagttttacgattaccgttcatcgattctcttgtttgctccagactctcaggcaatgacctgatagcctttgtagagacctctcaaaaatagctaccctctccggcatgaatttatcagctagaacggttgaatatcatattgatggtgatttgactgtctccggcctttctcacccgtttgaatctttacctacacattactcaggcattgcatttaaaatatatgagggttctaaaaatttttatccttgcgttgaaataaaggcttctcccgcaaaagtattacagggtcataatgtttttggtacaaccgatttagctttatgctctgaggctttattgcttaattttgctaattctttgccttgcctgtatgatttattggatgttggaatcgcctgatgcggtattttctccttacgcatctgtgcggtatttcacaccgcatatggtgcactctcagtacaatctgctctgatgccgcatagttaagccagccccgacacccgccaacacccgctgacgcgccctgacgggcttgtctgctcccggcatccgcttacagacaagctgtgaccgtctccgggagctgcatgtgtcagaggttttcaccgtcatcaccgaaacgcgcgagacgaaagggcctcgtgatacgcctatttttataggttaatgtcatgataataatggtttcttagacgtcaggtggcacttttcggggaaatgtgcgcggaacccctatttgtttatttttctaaatacattcaaatatgtatccgctcatgagacaataaccctgataaatgcttcaataatattgaaaaaggaagagtatgattgaacaagatggattgcacgcaggttctccggccgcttgggtggagaggctattcggctatgactgggcacaacagacaatcggctgctctgatgccgccgtgttccggctgtcagcgcaggggcgcccggttctttttgtcaagaccgacctgtccggtgccctgaatgaactgcaagacgaggcagcgcggctatcgtggctggccacgacgggcgttccttgcgcagctgtgctcgacgttgtcactgaagcgggaagggactggctgctattgggcgaagtgccggggcaggatctcctgtcatctcaccttgctcctgccgagaaagtatccatcatggctgatgcaatgcggcggctgcatacgcttgatccggctacctgcccattcgaccaccaagcgaaacatcgcatcgagcgagcacgtactcggatggaagccggtcttgtcgatcaggatgatctggacgaagagcatcaggggctcgcgccagccgaactgttcgccaggctcaaggcgagcatgcccgacggcgaggatctcgtcgtgacccatggcgatgcctgcttgccgaatatcatggtggaaaatggccgcttttctggattcatcgactgtggccggctgggtgtggcggaccgctatcaggacatagcgttggctacccgtgatattgctgaagagcttggcggcgaatgggctgaccgcttcctcgtgctttacggtatcgccgctcccgattcgcagcgcatcgccttctatcgccttcttgacgagttcttctgactgtcagaccaagtttactcatatatactttagattgatttaaaacttcatttttaatttaaaaggatctaggtgaagatcctttttgataatctcatgaccaaaatcccttaacgtgagttttcgttccactgagcgtcagaccccgtagaaaagatcaaaggatcttcttgagatcctttttttctgcgcgtaatctgctgcttgcaaacaaaaaaaccaccgctaccagcggtggtttgtttgccggatcaagagctaccaactctttttccgaaggtaactggcttcagcagagcgcagataccaaatactgttcttctagtgtagccgtagttaggccaccacttcaagaactctgtagcaccgcctacatacctcgctctgctaatcctgttaccagtggctgctgccagtggcgataagtcgtgtcttaccgggttggactcaagacgatagttaccggataaggcgcagcggtcgggctgaacggggggttcgtgcacacagcccagcttggagcgaacgacctacaccgaactgagatacctacagcgtgagctatgagaaagcgccacgcttcccgaagggagaaaggcggacaggtatccggtaagcggcagggtcggaacaggagagcgcacgagggagcttccagggggaaacgcctggtatctttatagtcctgtcgggtttcgccacctctgacttgagcgtcgatttttgtgatgctcgtcaggggggcggagcctatggaaaaacgccagcaacgcggcctttttacggttcctggccttttgctggccttttgctcacatgttctttcctgcgttatcccctgattctgtggataaccgtattaccgcctttgagtgagctgataccgctcgccgcagccgaacgaccgagcgcagcgagtcagtgagcgaggaagcggaagagcgcccaatacgcaaaccgcctctccccgcgcgttggccgattcattaatgcagctgcgcgctcgctcgctcactgaggccgcccgggcaaagcccgggcgtcgggcgacctttggtcgcccggcctcagtgagcgagcgagcgcgcagagagggagtggccaactccatcactaggggttccttgtagttaatgattaacccgccatgctacttatctacgtagccatgctctagcggcctcggcctctgcataaataaaaaaaattagtcagccatgagcttggcccattgcatacgttgtatccatatcataatatgtacatttatattggctcatgtccaacattac

SEQ ID NO: 4 - DNA, 9271 bp, synthetic construct
  source 1..9271: mol_type = other DNA
cgccatgttgacattgattattgactagttattaatagtaatcaattacggggtcattagttcatagcccatatatggagttccgcgttacataacttacggtaaatggcccgcctggctgaccgcccaacgacccccgcccattgacgtcaataatgacgtatgttcccatagtaacgccaatagggactttccattgacgtcaatgggtggagtatttacggtaaactgcccacttggcagtacatcaagtgtatcatatgccaagtacgccccctattgacgtcaatgacggtaaatggcccgcctggcattatgcccagtacatgaccttatgggactttcctacttggcagtacatctacgtattagtcatcgctattaccatggtgatgcggttttggcagtacatcaatgggcgtggatagcggtttgactcacggggatttccaagtctccaccccattgacgtcaatgggagtttgttttggcaccaaaatcaacgggactttccaaaatgtcgtaacaactccgccccattgacgcaaatgggcggtaggcgtgtacggtgggaggtctatataagcagagctcgtttagtgaaccgtcagatcgcctggagacgccatccacgctgttttgacctccatagaagacaccgggaccgatccagcctcccctcgaagcttacatgtggtaccatggcgaccgcagcgtctaaccactacagcctgctcacctccagcgcctccatcgtgcacgccgagccgcccggcggcatgcagcagggcgcggggggctaccgcgaagcgcagagcctggtgcagggcgactacggcgctctgcagagcaacggacacccgctcagccacgctcaccagtggatcaccgcgctgtcccacggcggcggcggcgggggcggtggcggcggcggggggggcgggggcggcggcgggggcggcggcgacggctccccgtggtccaccagccccctgggccagccggacatcaagccctcggtggtggtgcagcagggcggccgcggagacgagctgcacgggccaggcgccctgcagcagcagcatcagcagcagcaacagcaacagcagcagcaacagcagcaacagcagcagcagcagcagcaacagcggccgccgcatctggtgcaccacgccgctaaccaccacccgggacccggggcatggcggagcgcggcggctgcagcgcacctcccaccctccatgggagcgtccaacggcggcttgctctactcgcagcccagcttcacggtgaacggcatgctgggcgccggcgggcagccggccgggctgcaccaccacggcctgcgggacgcgcacgacgagccacaccatgccgaccaccacccgcacccgcactcgcacccacaccagcagccgccgcccccgccgcccccgcagggtccgcctggccacccaggcgcgcaccacgacccgcactcggacgaggacacgccgacctcggacgacctggagcagttcgccaagcagttcaagcagcggcggatcaaactgggatttacccaagcggacgtggggctggctctgggcaccctgtatggcaacgtgttctcgcagaccaccatctgcaggtttgaggccctgcagctgagcttcaagaacatgtgcaagctgaagcctttgttgaacaagtggttggaggaggcggactcgtcctcgggcagccccacgagcatagacaagatcgcagcgcaagggcgcaagcggaaaaagcggacctccatcgaggtgagcgtcaagggggctctggagagccatttcctcaaatgccccaagccctcggcccaggagatcacctccctcgcggacagcttacagctggagaaggaggtggtgagagtttggttttgtaacaggagacagaaagagaaaaggatgacccctcccggagggactctgccgggcgccgaggatgtgtacggggggagtagggacactccaccacaccacggggtgcagacgcccgtccagggtagcggtgccactaacttctccctgttgaaacaagcaggggatgtcgaagagaatcctggtccaatggaaaaatccaaaaatttccgcatcgacgccctgctggcggtggaccccccacgagccgcctctgcgcagagcgcgccgctggccttggtcacgtcgctcgccgccgccgcatctggcaccggaggtggcggcggcggcggcggggcgagcggcgggactagcggcagctgcagccccgcgtcctcggagccgccggctgcgcccgccgaccgcctgcgcgccgagagcccgtcgccgccgcgcctgctggccgcgcactgcgcgctgctgcccaagccgggcttcctgggcgcgggcggcggcggcggcggcacgggcggcgggcacggggggccccaccaccacgcgcatccgggcgcagcggccgctgccgccgccgccgccgccgccgccgccgctgggggcctggcgctggggctgcaccctgggggcgcgcagggcggcgcgggcctcccggcgcaggcggcgctctacggccacccggtctacggctactccgcggcggcggcggcggctgcgctggcgggccagcacccggcgctctcctactcgtacccgcaggtgcaaggcgcgcaccccgcgcaccccgccgaccccatcaagctgggcgccggcaccttccagctggaccagtggctgcgcgcgtccaccgcgggcatgatcctgcctaagatgcccgacttcaactcccaggcgcagtcgaacctcctggggaagtgccgccggccgcgcaccgccttcaccagccagcagctgctggagctggagcaccagttcaagctcaacaagtacctgtcgcggcccaagcgcttcgaggtggccacctcgctcatgctcaccgagacccaggtgaagatttggttccagaaccggcggatgaaatggaaacgcagcaaaaaggccaaagagcaggcggcgcaggaagcggagaaacagaagggcggcggcgggggcgcggggaagggcggcgcggaggagccgggagccgaggagctgctggggccgccagcgcccggagacaagggcagcggacgccgcctgcgggacttgagggacagtgaccccgaggaggacgaggacgaggacgacgaggaccatttcccctacagcaacggcgccagcgtccacgccgcctcctccgactgctcctcggaggacgactcgccgcccccgcggcccagccaccagcccgcgccccagggcagtggagagggcagaggaagtctgctaacatgcggtgacgtcgaggagaatcctggcccaatgaccaaatcgtacagcgagagtgggctgatgggcgagcctcagccccaaggtcctccaagctggacagacgagtgtctcagttctcaggacgaggagcacgaggcagacaagaaggaggacgacctcgaagccatgaacgcagaggaggactcactgaggaacgggggagaggaggaggacgaagatgaggacctggaagaggaggaagaagaggaagaggaggatgacgatcaaaagcccaagagacgcggccccaaaaagaagaagatgactaaggctcgcctggagcgttttaaattgagacgcatgaaggctaacgcccgggagcggaaccgcatgcacggactgaacgcggcgctagacaacctgcgcaaggtggtgccttgctattctaagacgcagaagctgtccaaaatcgagactctgcgcttggccaagaactacatctgggctctgtcggagatcctgcgctcaggcaaaagcccagacctggtctccttcgttcagacgctttgcaagggcttatcccaacccaccaccaacctggttgcgggctgcctgcaactcaatcctcggacttttctgcctgagcagaaccaggacatgcccccccacctgccgacggccagcgcttccttccctgtacacccctactcctaccagtcgcctgggctgcccagtccgccttacggtaccatggacagctcccatgtcttccacgttaagcctccgccgcacgcctacagcgcagcgctggagcccttctttgaaagccctctgactgattgcaccagcccttcctttgatggacccctcagcccgccgctcagcatcaatggcaacttctctttcaaacacgaaccgtccgccgagtttgagaaaaattatgcctttaccatgcactatcctgcagcgacactggcaggggcccaaagccacggatcaatcttctcaggcaccgctgcccctcgctgcgagatccccatagacaatattatgtccttcgatagccattcacatcatgagcgagtcatgagtgcccagctcaatgccatatttcatgattagcggccgctctagaggatccaagcttatcgataccgtcgacctcgagggcccagatctaattcaccccaccagtgcaggctgcctatcagaaagtggtggctggtgtggctaatgccctggcccacaagtatcactaagctcgctttcttgctgtccaatttctattaaaggttcctttgttccctaagtccaactactaaactgggggatattatgaagggccttgagcatctggattctgcctaataaaaaacatttattttcattgcaatgatgtatttaaattatttctgaatattttactaaaaagggaatgtgggaggtcagtgcatttaaaacataaagaaatgaagagctagttcaaaccttgggaaaatacactatatcttaaactccatgaaagaaggtgaggctgcaaacagctaatgcacattggcaacagcccctgatgcctatgccttattcatccctcagaaaaggattcaagtagaggcttgatttggaggttaaagttttgctatgctgtattttacattacttattgttttagctgtcctcatgaatgtcttttcactacccatttgcttatcctgcatctctcagccttgactccactcagttctcttgcttagagataccacctttcccctgaagtgttccttccatgttttacggcgagatggtttctcctcgcctggccactcagccttagttgtctctgttgtcttatagaggtctacttgaagaaggaaaaacagggggcatggtttgactgtcctgtgagcccttcttccctgcctcccccactcacagtgacccggaatccctcgacatctagagcatggctacgtagataagtagcatggcgggttaatcattaactacaaggaacccctagtgatggagttggccactccctctctgcgcgctcgctcgctcactgaggccgggcgaccaaaggtcgcccgacgcccgggctttgcccgggcggcctcagtgagcgagcgagcgcgcagctggcgtaatagcgaagaggcccgcaccgatcgcccttcccaacagttgcgcagcctgaatggcgaatggcgattccgttgcaatggctggcggtaatattgttctggatattaccagcaaggccgatagtttgagttcttctactcaggcaagtgatgttattactaatcaaagaagtattgcgacaacggttaatttgcgtgatggacagactcttttactcggtggcctcactgattataaaaacacttctcaggattctggcgtaccgttcctgtctaaaatccctttaatcggcctcctgtttagctcccgctctgattctaacgaggaaagcacgttatacgtgctcgtcaaagcaaccatagtacgcgccctgtagcggcgcattaagcgcggcgggtgtggtggttacgcgcagcgtgaccgctacacttgccagcgccctagcgcccgctcctttcgctttcttcccttcctttctcgccacgttcgccggctttccccgtcaagctctaaatcgggggctccctttagggttccgatttagtgctttacggcacctcgaccccaaaaaacttgattagggtgatggttcacgtagtgggccatcgccctgatagacggtttttcgccctttgacgttggagtccacgttctttaatagtggactcttgttccaaactggaacaacactcaaccctatctcggtctattcttttgatttataagggattttgccgatttcggcctattggttaaaaaatgagctgatttaacaaaaatttaacgcgaattttaacaaaatattaacgcttacaatttaaatatttgcttatacaatcttcctgtttttggggcttttctgattatcaaccggggtacatatgattgacatgctagttttacgattaccgttcatcgattctcttgtttgctccagactctcaggcaatgacctgatagcctttgtagagacctctcaaaaatagctaccctctccggcatgaatttatcagctagaacggttgaatatcatattgatggtgatttgactgtctccggcctttctcacccgtttgaatctttacctacacattactcaggcattgcatttaaaatatatgagggttctaaaaatttttatccttgcgttgaaataaaggcttctcccgcaaaagtattacagggtcataatgtttttggtacaaccgatttagctttatgctctgaggctttattgcttaattttgctaattctttgccttgcctgtatgatttattggatgttggaatcgcctgatgcggtattttctccttacgcatctgtgcggtatttcacaccgcatatggtgcactctcagtacaatctgctctgatgccgcatagttaagccagccccgacacccgccaacacccgctgacgcgccctgacgggcttgtctgctcccggcatccgcttacagacaagctgtgaccgtctccgggagctgcatgtgtcagaggttttcaccgtcatcaccgaaacgcgcgagacgaaagggcctcgtgatacgcctatttttataggttaatgtcatgataataatggtttcttagacgtcaggtggcacttttcggggaaatgtgcgcggaacccctatttgtttatttttctaaatacattcaaatatgtatccgctcatgagacaataaccctgataaatgcttcaataatattgaaaaaggaagagtatgattgaacaagatggattgcacgcaggttctccggccgcttgggtggagaggctattcggctatgactgggcacaacagacaatcggctgctctgatgccgccgtgttccggctgtcagcgcaggggcgcccggttctttttgtcaagaccgacctgtccggtgccctgaatgaactgcaagacgaggcagcgcggctatcgtggctggccacgacgggcgttccttgcgcagctgtgctcgacgttgtcactgaagcgggaagggactggctgctattgggcgaagtgccggggcaggatctcctgtcatctcaccttgctcctgccgagaaagtatccatcatggctgatgcaatgcggcggctgcatacgcttgatccggctacctgcccattcgaccaccaagcgaaacatcgcatcgagcgagcacgtactcggatggaagccggtcttgtcgatcaggatgatctggacgaagagcatcaggggctcgcgccagccgaactgttcgccaggctcaaggcgagcatgcccgacggcgaggatctcgtcgtgacccatggcgatgcctgcttgccgaatatcatggtggaaaatggccgcttttctggattcatcgactgtggccggctgggtgtggcggaccgctatcaggacatagcgttggctacccgtgatattgctgaagagcttggcggcgaatgggctgaccgcttcctcgtgctttacggtatcgccgctcccgattcgcagcgcatcgccttctatcgccttcttgacgagttcttctgactgtcagaccaagtttactcatatatactttagattgatttaaaacttcatttttaatttaaaaggatctaggtgaagatcctttttgataatctcatgaccaaaatcccttaacgtgagttttcgttccactgagcgtcagaccccgtagaaaagatcaaaggatcttcttgagatcctttttttctgcgcgtaatctgctgcttgcaaacaaaaaaaccaccgctaccagcggtggtttgtttgccggatcaagagctaccaactctttttccgaaggtaactggcttcagcagagcgcagataccaaatactgttcttctagtgtagccgtagttaggccaccacttcaagaactctgtagcaccgcctacatacctcgctctgctaatcctgttaccagtggctgctgccagtggcgataagtcgtgtcttaccgggttggactcaagacgatagttaccggataaggcgcagcggtcgggctgaacggggggttcgtgcacacagcccagcttggagcgaacgacctacaccgaactgagatacctacagcgtgagctatgagaaagcgccacgcttcccgaagggagaaaggcggacaggtatccggtaagcggcagggtcggaacaggagagcgcacgagggagcttccagggggaaacgcctggtatctttatagtcctgtcgggtttcgccacctctgacttgagcgtcgatttttgtgatgctcgtcaggggggcggagcctatggaaaaacgccagcaacgcggcctttttacggttcctggccttttgctggccttttgctcacatgttctttcctgcgttatcccctgattctgtggataaccgtattaccgcctttgagtgagctgataccgctcgccgcagccgaacgaccgagcgcagcgagtcagtgagcgaggaagcggaagagcgcccaatacgcaaaccgcctctccccgcgcgttggccgattcattaatgcagctgcgcgctcgctcgctcactgaggccgcccgggcaaagcccgggcgtcgggcgacctttggtcgcccggcctcagtgagcgagcgagcgcgcagagagggagtggccaactccatcactaggggttccttgtagttaatgattaacccgccatgctacttatctacgtagccatgctctagcggcctcggcctctgcataaataaaaaaaattagtcagccatgagcttggcccattgcatacgttgtatccatatcataatatgtacatttatattggctcatgtccaacattac

SEQ ID NO: 5 - DNA, 9827 bp, synthetic construct
  source 1..9827: mol_type = other DNA
cgccatgttgacattgattattgactagttattaatagtaatcaattacggggtcattagttcatagcccatatatggagttccgcgttacataacttacggtaaatggcccgcctggctgaccgcccaacgacccccgcccattgacgtcaataatgacgtatgttcccatagtaacgccaatagggactttccattgacgtcaatgggtggagtatttacggtaaactgcccacttggcagtacatcaagtgtatcatatgccaagtacgccccctattgacgtcaatgacggtaaatggcccgcctggcattatgcccagtacatgaccttatgggactttcctacttggcagtacatctacgtattagtcatcgctattaccatggtgatgcggttttggcagtacatcaatgggcgtggatagcggtttgactcacggggatttccaagtctccaccccattgacgtcaatgggagtttgttttggcaccaaaatcaacgggactttccaaaatgtcgtaacaactccgccccattgacgcaaatgggcggtaggcgtgtacggtgggaggtctatataagcagagctcgtttagtgaaccgtcagatcgcctggagacgccatccacgctgttttgacctccatagaagacaccgggaccgatccagcctcccctcgaagcttacatgtggtaccatggcagcaaggcccaagctccactatcccaacggaagaggccggatggagtccgtgagatgggttttagctgccgccggagtcgagtttgatgaagaatttctggaaacaaaagaacagttgtacaagttgcaggatggtaaccacctgctgttccaacaagtgcccatggttgaaattgacgggatgaagttggtacagacccgaagcattctccactacatagcagacaagcacaatctctttggcaagaacctcaaggagagaaccctgattgacatgtacgtggaggggacactggatctgctggaactgcttatcatgcatcctttcttaaaaccagatgatcagcaaaaggaagtggttaacatggcccagaaggctataattagatactttcctgtgtttgaaaagattttaaggggtcacggacaaagctttcttgttggtaatcagctgagccttgcagatgtgattttactccaaaccattttagctctagaagagaaaattcctaatatcctgtctgcatttcctttcctccaggaatacacagtgaaactaagtaatatccctacaattaagagattccttgaacctggcagcaagaagaagcctccccctgatgaaatttatgtgagaaccgtctacaacatctttaggccaggtagcggtgccactaacttctccctgttgaaacaagcaggggatgtcgaagagaatcctggtccaatggaggtggacaccgaggagaagcggcatcgcacgcggtccaaaggggttcgagttcccgtggaaccagccatacaagagctgttcagctgtcccacccctggctgtgacggcagtggtcatgtcagtggcaaatatgcaagacacagaagtgtatatggttgtcccttggcgaaaaaaagaaaaacacaagataaacagccccaggaacctgctcctaaacgaaagccatttgccgtgaaagcagacagctcctcagtggatgagtgtgacgacagtgatgggactgaggacatggatgagaaggaggaggatgagggggaggagtactccgaggacaatgacgagccaggggatgaggacgaggaggacgaggagggggaccgggaggaggaggaggagatcgaggaggaggatgaggacgatgacgaggatggagaagatgtggaggatgaagaagaggaagaggaggaggaggaggaggaggaagaggaagaagaaaacgaagaccatcaaatgaattgtcacaatactcgaataatgcaagacacagaaaaggatgataacaataatgacgaatatgacaattacgatgaactggtggccaagtcattgttaaacctcggcaaaatcgctgaggatgcagcctaccgggccaggactgagtcagaaatgaacagcaatacctccaatagtctggaagacgatagtgacaaaaacgaaaacctgggtcggaaaagtgagttgagtttagacttagacagtgatgttgttagagaaacagtggactcccttaaactattagcccaaggacacggtgttgtgctctcagaaaacatgaatgacagaaattatgcagacagcatgtcgcagcaagacagtagaaatatgaattacgtcatgttggggaagcccatgaacaatggactcatggaaaagatggtggaggagagcgatgaggaggtgtgtctgagcagtctggagtgtttgaggaatcagtgcttcgacctggccaggaagctcagtgagaccaacccgcaggagaggaatccgcagcagaacatgaacatccgtcagcatgtccggccagaagaggacttcccaggaaggacgccggacagaaactactcggacatgctgaacctcatgcggctggaggagcagttgagcccccggtcgagagtgtttgccagctgtgcgaaggaggatgggtgtcatgagcgggacgacgataccacctctgtgaactcggacaggtctgaagaggtgttcgacatgaccaaggggaacctgaccctgctggagaaagccatcgctttggaaacggaaagagcaaaggccatgagggagaagatggccatggaagctgggaggagggacaatatgaggtcatatgaggaccagtctccgagacaacttcccggggaggacagaaagcctaaatccagtgacagccatgtcaaaaagccatactatgatccctcaagaacagaaaagaaagagagcaagtgtccaacccccgggtgtgatggaaccggccacgtaactgggctgtacccacatcaccgcagcctgtccggatgcccgcacaaagatagggtccctccagaaatccttgccatgcatgaaagtgtcctcaagtgccccactccgggctgcacggggcgcgggcatgtcaacagcaacaggaactcccaccgaagcctctccggatgcccgatcgctgcagcagagaaactggccaaggcacaggaaaagcaccagagctgcgacgtgtccaagtccagccaggcctcggaccgcgtgctcaggccaatgtgctttgtgaagcagctggagattcctcagtatggctacagaaacaatgtccccacaactacgccgcgttccaacctggccaaggagctcgagaaatattccaagacctcgtttgaatacaacagttacgacaaccatacttatggcaagcgagccatagctcccaaggtgcaaaccagggatatatcccccaaaggatatgatgatgcgaagcggtactgcaaggaccccagccccagcagcagcagcaccagcagctacgcgcccagcagcagcagcaacctgagctgcggcgggggcagcagcgccagcagcacgtgcagcaagagcagcttcgactacacgcacgacatggaggcggcccacatggcggccaccgccatcctcaacctgtccacgcgctgccgcgagatgccgcagaacctgagcaccaagccgcaggacctgtgcgccacgcggaaccctgacatggaggtggatgagaacgggaccctggacctcagcatgaacaagcagaggccgcgggacagctgctgccccatcctgacccctctggagcccatgtccccccagcagcaggcagtgatgaacaaccggtgtttccagctgggcgagggcgactgctgggacttgcccgtagactacaccaaaatgaaaccccggaggatagacgaggacgagtccaaagacattactccagaagacttggacccattccaggaggctctagaagaaagacggtatcccggggaggtgaccatcccaagtcccaaacccaagtaccctcagtgcaaggagagcaaaaaggacttaataactctgtctggctgccccctggcggacaaaagcattcgaagtatgctggccaccagctcccaagaactcaagtgccccacgcctggctgtgatggttctggacatatcaccggcaattatgcttctcatcggagcctttcaggttgcccaagagcaaagaaaagtggtatcaggatagcacagagcaaagaagataaagaagatcaagaacccatcaggtgtccggtccccgggtgcgacggccagggccacatcactgggaagtacgcgtcccatcgcagcgcctccgggtgccccttggcggccaagaggcagaaagacgggtacctgaatggctcccagttctcctggaagtcggtcaagacggaaggcatgtcctgccccacgccaggatgcgacggctcaggccacgtcagcggcagcttcctcacacaccgcagcttgtcaggatgcccgagagccacgtcagcgatgaagaaggcaaagctttctggagagcagatgctgaccatcaaacagcgggccagcaacggtatagaaaatgatgaagaaatcaaacagttagatgaagaaatcaaggagctaaatgaatccaattcccagatggaagccgatatgattaaactcagaactcagattaccacgatggagagcaacctgaagaccatcgaagaggagaacaaagtgattgagcagcagaacgagtctctcctccacgagctggcgaacctgagccagtctctgatccacagcctggctaacatccagctgccgcacatggatccaatcaatgaacaaaattttgatgcttacgtgactactttgacggaaatgtatacaaatcaagatcgttatcagagtccagaaaataaagccctactggaaaatataaagcaggctgtgagaggaattcaggtctgagcggccgctctagaggatccaagcttatcgataccgtcgacctcgagggcccagatctaattcaccccaccagtgcaggctgcctatcagaaagtggtggctggtgtggctaatgccctggcccacaagtatcactaagctcgctttcttgctgtccaatttctattaaaggttcctttgttccctaagtccaactactaaactgggggatattatgaagggccttgagcatctggattctgcctaataaaaaacatttattttcattgcaatgatgtatttaaattatttctgaatattttactaaaaagggaatgtgggaggtcagtgcatttaaaacataaagaaatgaagagctagttcaaaccttgggaaaatacactatatcttaaactccatgaaagaaggtgaggctgcaaacagctaatgcacattggcaacagcccctgatgcctatgccttattcatccctcagaaaaggattcaagtagaggcttgatttggaggttaaagttttgctatgctgtattttacattacttattgttttagctgtcctcatgaatgtcttttcactacccatttgcttatcctgcatctctcagccttgactccactcagttctcttgcttagagataccacctttcccctgaagtgttccttccatgttttacggcgagatggtttctcctcgcctggccactcagccttagttgtctctgttgtcttatagaggtctacttgaagaaggaaaaacagggggcatggtttgactgtcctgtgagcccttcttccctgcctcccccactcacagtgacccggaatccctcgacatctagagcatggctacgtagataagtagcatggcgggttaatcattaactacaaggaacccctagtgatggagttggccactccctctctgcgcgctcgctcgctcactgaggccgggcgaccaaaggtcgcccgacgcccgggctttgcccgggcggcctcagtgagcgagcgagcgcgcagctggcgtaatagcgaagaggcccgcaccgatcgcccttcccaacagttgcgcagcctgaatggcgaatggcgattccgttgcaatggctggcggtaatattgttctggatattaccagcaaggccgatagtttgagttcttctactcaggcaagtgatgttattactaatcaaagaagtattgcgacaacggttaatttgcgtgatggacagactcttttactcggtggcctcactgattataaaaacacttctcaggattctggcgtaccgttcctgtctaaaatccctttaatcggcctcctgtttagctcccgctctgattctaacgaggaaagcacgttatacgtgctcgtcaaagcaaccatagtacgcgccctgtagcggcgcattaagcgcggcgggtgtggtggttacgcgcagcgtgaccgctacacttgccagcgccctagcgcccgctcctttcgctttcttcccttcctttctcgccacgttcgccggctttccccgtcaagctctaaatcgggggctccctttagggttccgatttagtgctttacggcacctcgaccccaaaaaacttgattagggtgatggttcacgtagtgggccatcgccctgatagacggtttttcgccctttgacgttggagtccacgttctttaatagtggactcttgttccaaactggaacaacactcaaccctatctcggtctattcttttgatttataagggattttgccgatttcggcctattggttaaaaaatgagctgatttaacaaaaatttaacgcgaattttaacaaaatattaacgcttacaatttaaatatttgcttatacaatcttcctgtttttggggcttttctgattatcaaccggggtacatatgattgacatgctagttttacgattaccgttcatcgattctcttgtttgctccagactctcaggcaatgacctgatagcctttgtagagacctctcaaaaatagctaccctctccggcatgaatttatcagctagaacggttgaatatcatattgatggtgatttgactgtctccggcctttctcacccgtttgaatctttacctacacattactcaggcattgcatttaaaatatatgagggttctaaaaatttttatccttgcgttgaaataaaggcttctcccgcaaaagtattacagggtcataatgtttttggtacaaccgatttagctttatgctctgaggctttattgcttaattttgctaattctttgccttgcctgtatgatttattggatgttggaatcgcctgatgcggtattttctccttacgcatctgtgcggtatttcacaccgcatatggtgcactctcagtacaatctgctctgatgccgcatagttaagccagccccgacacccgccaacacccgctgacgcgccctgacgggcttgtctgctcccggcatccgcttacagacaagctgtgaccgtctccgggagctgcatgtgtcagaggttttcaccgtcatcaccgaaacgcgcgagacgaaagggcctcgtgatacgcctatttttataggttaatgtcatgataataatggtttcttagacgtcaggtggcacttttcggggaaatgtgcgcggaacccctatttgtttatttttctaaatacattcaaatatgtatccgctcatgagacaataaccctgataaatgcttcaataatattgaaaaaggaagagtatgattgaacaagatggattgcacgcaggttctccggccgcttgggtggagaggctattcggctatgactgggcacaacagacaatcggctgctctgatgccgccgtgttccggctgtcagcgcaggggcgcccggttctttttgtcaagaccgacctgtccggtgccctgaatgaactgcaagacgaggcagcgcggctatcgtggctggccacgacgggcgttccttgcgcagctgtgctcgacgttgtcactgaagcgggaagggactggctgctattgggcgaagtgccggggcaggatctcctgtcatctcaccttgctcctgccgagaaagtatccatcatggctgatgcaatgcggcggctgcatacgcttgatccggctacctgcccattcgaccaccaagcgaaacatcgcatcgagcgagcacgtactcggatggaagccggtcttgtcgatcaggatgatctggacgaagagcatcaggggctcgcgccagccgaactgttcgccaggctcaaggcgagcatgcccgacggcgaggatctcgtcgtgacccatggcgatgcctgcttgccgaatatcatggtggaaaatggccgcttttctggattcatcgactgtggccggctgggtgtggcggaccgctatcaggacatagcgttggctacccgtgatattgctgaagagcttggcggcgaatgggctgaccgcttcctcgtgctttacggtatcgccgctcccgattcgcagcgcatcgccttctatcgccttcttgacgagttcttctgactgtcagaccaagtttactcatatatactttagattgatttaaaacttcatttttaatttaaaaggatctaggtgaagatcctttttgataatctcatgaccaaaatcccttaacgtgagttttcgttccactgagcgtcagaccccgtagaaaagatcaaaggatcttcttgagatcctttttttctgcgcgtaatctgctgcttgcaaacaaaaaaaccaccgctaccagcggtggtttgtttgccggatcaagagctaccaactctttttccgaaggtaactggcttcagcagagcgcagataccaaatactgttcttctagtgtagccgtagttaggccaccacttcaagaactctgtagcaccgcctacatacctcgctctgctaatcctgttaccagtggctgctgccagtggcgataagtcgtgtcttaccgggttggactcaagacgatagttaccggataaggcgcagcggtcgggctgaacggggggttcgtgcacacagcccagcttggagcgaacgacctacaccgaactgagatacctacagcgtgagctatgagaaagcgccacgcttcccgaagggagaaaggcggacaggtatccggtaagcggcagggtcggaacaggagagcgcacgagggagcttccagggggaaacgcctggtatctttatagtcctgtcgggtttcgccacctctgacttgagcgtcgatttttgtgatgctcgtcaggggggcggagcctatggaaaaacgccagcaacgcggcctttttacggttcctggccttttgctggccttttgctcacatgttctttcctgcgttatcccctgattctgtggataaccgtattaccgcctttgagtgagctgataccgctcgccgcagccgaacgaccgagcgcagcgagtcagtgagcgaggaagcggaagagcgcccaatacgcaaaccgcctctccccgcgcgttggccgattcattaatgcagctgcgcgctcgctcgctcactgaggccgcccgggcaaagcccgggcgtcgggcgacctttggtcgcccggcctcagtgagcgagcgagcgcgcagagagggagtggccaactccatcactaggggttccttgtagttaatgattaacccgccatgctacttatctacgtagccatgctctagcggcctcggcctctgcataaataaaaaaaattagtcagccatgagcttggcccattgcatacgttgtatccatatcataatatgtacatttatattggctcatgtccaacattac

SEQ ID NO: 6 - DNA, 20 bp, synthetic construct
  source 1..20: mol_type = other DNA
gtggcactgaccaagacgta

SEQ ID NO: 7 - DNA, 20 bp, synthetic construct
  source 1..20: mol_type = other DNA
ctgacgtcctcatgtaggcc

SEQ ID NO: 8 - DNA, 20 bp, synthetic construct
  source 1..20: mol_type = other DNA
tcctccattctccctcctcg

SEQ ID NO: 9 - DNA, 20 bp, synthetic construct
  source 1..20: mol_type = other DNA
cgaattggctctgacctggt

SEQ ID NO: 10 - DNA, 20 bp, synthetic construct
  source 1..20: mol_type = other DNA
gagcttgaactggtgctcca

SEQ ID NO: 11 - DNA, 20 bp, synthetic construct
  source 1..20: mol_type = other DNA
tctcaacagtaggtgcctgc

SEQ ID NO: 12 - DNA, 669 bp, synthetic construct
  source 1..669: mol_type = other DNA
atggcagcaaggcccaagctccactatcccaacggaagaggccggatggagtccgtgagatgggttttagctgccgccggagtcgagtttgatgaagaatttctggaaacaaaagaacagttgtacaagttgcaggatggtaaccacctgctgttccaacaagtgcccatggttgaaattgacgggatgaagttggtacagacccgaagcattctccactacatagcagacaagcacaatctctttggcaagaacctcaaggagagaaccctgattgacatgtacgtggaggggacactggatctgctggaactgcttatcatgcatcctttcttaaaaccagatgatcagcaaaaggaagtggttaacatggcccagaaggctataattagatactttcctgtgtttgaaaagattttaaggggtcacggacaaagctttcttgttggtaatcagctgagccttgcagatgtgattttactccaaaccattttagctctagaagagaaaattcctaatatcctgtctgcatttcctttcctccaggaatacacagtgaaactaagtaatatccctacaattaagagattccttgaacctggcagcaagaagaagcctccccctgatgaaatttatgtgagaaccgtctacaacatctttaggccataa

SEQ ID NO: 13 - protein, 401 aa, synthetic construct
MEKSKNFRIDALLAVDPPRAASAQSAPLALVTSLAAAASGTGGGGGGGGASGGTSGSCSPASSEPPAAPADRLRAESPSPPRLLAAHCALLPKPGFLGAGGGGGGTGGGHGGPHHHAHPGAAAAAAAAAAAAAAGGLALGLHPGGAQGGAGLPAQAALYGHPVYGYSAAAAAAALAGQHPALSYSYPQVQGAHPAHPADPIKLGAGTFQLDQWLRASTAGMILPKMPDFNSQAQSNLLGKCRRPRTAFTSQQLLELEHQFKLNKYLSRPKRFEVATSLMLTETQVKIWFQNRRMKWKRSKKAKEQAAQEAEKQKGGGGGAGKGGAEEPGAEELLGPPAPGDKGSGRRLRDLRDSDPEEDEDEDDEDHFPYSNGASVHAASSDCSSEDDSPPPRPSHQPAPQ

SEQ ID NO: 14 - DNA, 1203 bp, synthetic construct
  source 1..1203: mol_type = other DNA
atggaaaaatccaaaaatttccgcatcgacgccctgctggcggtggaccccccacgagccgcctctgcgcagagcgcgccgctggccttggtcacgtcgctcgccgccgccgcatctggcaccggaggtggcggcggcggcggcggggcgagcggcgggactagcggcagctgcagccccgcgtcctcggagccgccggctgcgcccgccgaccgcctgcgcgccgagagcccgtcgccgccgcgcctgctggccgcgcactgcgcgctgctgcccaagccgggcttcctgggcgcgggcggcggcggcggcggcacgggcggcgggcacggggggccccaccaccacgcgcatccgggcgcagcggccgctgccgccgccgccgccgccgccgccgccgctgggggcctggcgctggggctgcaccctgggggcgcgcagggcggcgcgggcctcccggcgcaggcggcgctctacggccacccggtctacggctactccgcggcggcggcggcggctgcgctggcgggccagcacccggcgctctcctactcgtacccgcaggtgcaaggcgcgcaccccgcgcaccccgccgaccccatcaagctgggcgccggcaccttccagctggaccagtggctgcgcgcgtccaccgcgggcatgatcctgcctaagatgcccgacttcaactcccaggcgcagtcgaacctcctggggaagtgccgccggccgcgcaccgccttcaccagccagcagctgctggagctggagcaccagttcaagctcaacaagtacctgtcgcggcccaagcgcttcgaggtggccacctcgctcatgctcaccgagacccaggtgaagatttggttccagaaccggcggatgaaatggaaacgcagcaaaaaggccaaagagcaggcggcgcaggaagcggagaaacagaagggcggcggcgggggcgcggggaagggcggcgcggaggagccgggagccgaggagctgctggggccgccagcgcccggagacaagggcagcggacgccgcctgcgggacttgagggacagtgaccccgaggaggacgaggacgaggacgacgaggaccatttcccctacagcaacggcgccagcgtccacgccgcctcctccgactgctcctcggaggacgactcgccgcccccgcggcccagccaccagcccgcgccccag

SEQ ID NO: 15 - protein, 402 aa, synthetic construct
MEARGELGPARESAGGDLLLALLARRADLRREIPLCAGCDQHILDRFILKALDRHWHSKCLKCSDCHTPLAERCFSRGESVYCKDDFFKRFGTKCAACQLGIPPTQVVRRAQDFVYHLHCFACVVCKRQLATGDEFYLMEDSRLVCKADYETAKQREAEATAKRPRTTITAKQLETLKSAYNTSPKPARHVREQLSSETGLDMRVVQVWFQNRRAKEKRLKKDAGRQRWGQYFRNMKRSRGGSKSDKDSVQEGQDSDAEVSFPDEPSLAEMGPANGLYGSLGEPTQALGRPSGALGNFSLEHGGLAGPEQYRELRPGSPYGVPPSPAAPQSLPGPQPLLSSLVYPDTSLGLVPSGAPGGPPPMRVLAGNGPSSDLSTGSSGGYPDFPASPASWLDEVDHAQF

SEQ ID NO: 16 - DNA, 1206 bp, synthetic construct
  source 1..1206: mol_type = other DNA
atggaagccagaggcgaactgggccctgccagagaatctgccggcggagatctgctgctggccctgctggctagaagggccgacctgagaagagaaatccccctgtgcgccggctgcgaccagcacatcctggaccggtttatcctgaaggccctggacagacactggcacagcaagtgcctgaagtgcagcgactgccacacccccctggccgagagatgctttagcagaggcgagagcgtgtactgcaaggacgacttcttcaagagattcggcaccaagtgcgccgcctgccagctgggaattcctcctacacaggtcgtgcggagagcccaggacttcgtgtaccatctgcactgcttcgcctgcgtcgtgtgcaagagacagctggccaccggcgacgagttctacctgatggaagatagccggctcgtgtgtaaagccgactacgagacagccaagcagagagaggccgaggccaccgccaaaagacccagaaccaccatcaccgccaagcagctggaaaccctgaagtccgcctacaacaccagccccaagcccgccagacatgtgcgggaacagctgagcagcgagacaggcctggacatgagagtggtgcaagtgtggttccagaacagacgggccaaagagaagcggctgaagaaggacgccggcaggcagagatggggccagtacttccggaacatgaagcggtccagaggcggcagcaagagcgacaaggacagcgtgcaggaaggccaggacagcgacgccgaggtgtccttcccagatgagcctagcctggccgaaatgggcccagccaatggcctgtatggcagcctgggagagccaacccaggctctgggcagaccttctggcgccctgggcaacttctctctggaacacggcggactggccggacccgagcagtatagagaactgaggcccggcagcccttacggcgtgccaccttctccagctgcccctcagtctctgccaggacctcagcctctgctgtccagcctggtgtaccccgatacaagcctgggcctggtgccatctggcgctccaggcggacctcctccaatgagagtgctggccggcaatggccctagcagcgatctgagcacaggcagctctggcggctaccccgattttcctgccagccctgcctcctggctggacgaagtggatcacgcccagttc

SEQ ID NO: 17 - protein, 231 aa, synthetic construct
MESSGKMESGAGQQPQPPQPFLPPAACFFATAAAAAAAAAAAAQSAQQQQPQAPPQQAPQLSPVADSQPSGGGHKSAAKQVKRQRSSSPELMRCKRRLNFSGFGYSLPQQQPAAVARRNERERNRVKLVNLGFATLREHVPNGAANKKMSKVETLRSAVEYIRALQQLLDEHDAVSAAFQAGVLSPTISPNYSNDLNSMAGSPVSSYSSDEGSYDPLSPEEQELLDFTNWF

SEQ ID NO: 18 - DNA, 696 bp, synthetic construct
  source 1..696: mol_type = other DNA
atggagagctctggcaagatggagagtggagccggccagcagccgcagcccccgcagcccttcctgcctcccgcagcctgcttctttgcgaccgcggcggcggcggcagcggcggcggccgcggcagctcagagcgcgcagcagcaacagccgcaggcgccgccgcagcaggcgccgcagctgagcccggtggccgacagccagccctcagggggcggtcacaagtcagcggccaagcaggtcaagcgccagcgctcgtcctctccggaactgatgcgctgcaaacgccggctcaacttcagcggcttcggctacagcctgccacagcagcagccggccgccgtggcgcgccgcaacgagcgcgagcgcaaccgggtcaagttggtcaacctgggttttgccaccctccgggagcatgtccccaacggcgcggccaacaagaagatgagcaaggtggagacgctgcgctcggcggtcgagtacatccgcgcgctgcagcagctgctggacgagcacgacgcggtgagcgctgcctttcaggcgggcgtcctgtcgcccaccatctcccccaactactccaacgacttgaactctatggcgggttctccggtctcgtcctactcctccgacgagggatcctacgaccctcttagcccagaggaacaagagctgctggactttaccaactggttctga

SEQ ID NO: 19 - protein, 284 aa, synthetic construct
MATAASNHYSTSSASVHAGGMGAGGYRASVGDYGASNGHSHAHWTASHGGGGGGGGGGGGGGGGGGGGGDGSWSTSGDKSVVVGGRGDHGGAHRHVHHAANHHGGAWRSAAAAAHSMGASNGGYSSTVNGMGAGGAGHHHGRDAHDHHADHHHHSHHGGHGAHHDHSDDTTSDDAKKRRKGTADVGAGTYGNVSTTCRASKNMCKKNKWADSSSGSTSDKAAGRKRKKRTSVSVKGASHKCKSATSADSKVVRVWCNRRKKRMTGGTGADVYGGSRDTHHGVTV

SEQ ID NO: 20 - DNA, 1338 bp, synthetic construct
  source 1..1338: mol_type = other DNA
atggcgaccgcagcgtctaaccactacagcctgctcacctccagcgcctccatcgtacatgccgagccgcctggcggcatgcagcagggcgcagggggctaccgcgaggcgcagagcctggtgcagggcgactacggcgcgctgcagagcaacgggcacccgctcagccacgctcaccagtggatcaccgcgctgtcccacggcggcggcggcgggggcggcggcggcggtggaggaggcgggggaggcggcgggggaggcggcgacggctccccgtggtccaccagccccctaggccagccggacatcaagccctcggtggtggtacagcagggtggccgaggcgacgagctgcacgggccaggagcgctgcagcaacagcatcaacagcaacagcaacagcagcagcagcagcagcagcagcagcagcagcaacagcagcagcaacaacagcgaccgccacatctggtgcaccacgctgccaaccaccatcccgggcccggggcatggcggagtgcggcggctgcagctcacctccctccctccatgggagcttccaacggcggtttgctctattcgcagccgagcttcacggtgaacggcatgctgggcgcaggagggcagccggctgggctgcaccaccacggcctgagggacgcccacgatgagccacaccatgcagaccaccacccgcatccgcactctcacccacaccagcaaccgcccccgccacctcccccacaaggcccaccgggccacccaggcgcgcaccacgacccgcactcggacgaggacacgccgacctcagacgacctggagcagttcgccaagcaattcaagcagaggcggatcaaactcggatttactcaagcagacgtggggctggcgcttggcaccctgtacggcaacgtgttctcgcagaccaccatctgcaggtttgaggccctgcagctgagcttcaagaacatgtgcaagctgaagcctttgttgaacaagtggttggaagaggcagactcatcctcgggcagccccaccagcatagacaagatcgcagcgcaagggcgcaaacggaaaaagcggacctccatcgaggtgagcgtcaagggggctctggagagccatttcctcaaatgccctaagccctcggcccaggagatcacctccctcgcggacagcttacagctggagaaggaggtggtgagagtttggttttgtaacaggagacagaaagagaaaaggatgacccctcccggagggactctgccgggcgccgaggatgtgtatgggggtagtagggacacgccaccacaccacggggtgcagacgcccgtccagtga

SEQ ID NO: 21 - protein, 813 aa, synthetic construct
MDVDSKRHRTRSKGVRVVASCTGCDGSGHVSGKYARHRSVYGCAKKRKTDKAKRKAVKADSSSVDCYSDGTDMDDKDDDSDNDGDDDDDVDRDDDDDDDDGDDVDDDNDHMSCTRMDTDKDDNNNDYDNYDVAKSNGKADAAYRARTSMNSNTSNSDDSDKNNGRKSSDDSDVVRTVDSKAGHGVVSNSDRSYAGMSDSRNMNYVMGKMNNGMKMVSDVCSSCRNCDARKSTNDRSNMSVRHVRDDGRTDRSYSDMMNMRSRSRTSSCAKDGCHRDDDTTSVNSDRSVDMTKGNTKAATRAKAMRKMAMDAGRRDNRSYDSRAGDRKSKSSDSHVKKYYGKDSRTKRSKCTGCDGTGHVTGYHHRSSGCHKDRVAMHNVKCTGCTGRGHVNSNRNSHRSSGCAAAKAKAKHSCDVSKSNASDRVRMCVKYGYRNNVTTTRSNAKKYSKTSYNSYDNHTYGKRAAKVTRDSKGYDDAKRYCKNASSSSTTSSYASSSSNSCGGGSSASSTCSKSSDYTHDMAAHMAATANSTRCRMNSTKDCTARNDMVDNGTDSMNKRRDSCCVTMSAVMSSRCSGDCWDVDYTKMKRRVDDKTDDARRYGVTSKKYCKSKKDTSGCADKSRSMATSSKCTGCDGSGHTGNYASHRSSGCRAKKSGRASKDKDRCVGCDGGHTGKYASHRSASGCAAKRKDGYNGSSWKSVKTGMSCTGCDGSGHVSGSTHRSSGCRATSAMKKAKSGMTKRASNGNDKDKNSNSMADMKRTTTMSNKTNKVNSHANSSHSANHMDNNDAYVTTTMYTNDRYSNKANKAVRGV

SEQ ID NO: 22 - DNA, 3564 bp, synthetic construct
  source 1..3564: mol_type = other DNA
atggacgtggactctgaggagaagcgccatcgcacacggtccaaaggggttcgagttcctgtggagccagccatacaagagctgttcagctgtcccactccaggctgcgacggcagtggtcacgtcagtggcaaatatgcacgacacagaagtgtatatggttgtcccttggctaaaaaaagaaaaacgcaagataaacagccccaagaacctgctcccaagcgaaaaccatttgcagtaaaagcagatagttcctcagtagacgaatgttatgagagtgatggtactgaagacatggatgataaggaggaagatgatgatgaggagttctctgaagacaatgatgagcaaggggatgatgacgacgaagatgaggtggatcgggaagacgaggaggagatcgaggaggaagatgatgaagaagatgatgatgatgaagatggtgacgatgtagaagaggaagaagaggatgatgatgaagaggaggaagaagaggaagaggaagaagaaaatgaagaccatcaaatgagttgtactcgaataatgcaggacacagacaaggatgataacaacaatgatgagtatgataactatgatgaactggtagctaagtcgctattaaatcttggcaaaattgctgaggatgcagcataccgagccaggactgaatcagagatgaacagcaatacctccaatagtctggaggacgatagtgacaaaaacgaaaacctcggtcggaaaagcgaactgagtctagacttagacagtgatgttgttagagaaacagtggactcccttaagctgttagcacaaggacatggtgttgtgctatcagagaatatcagtgacagaagttatgctgaggggatgtcacagcaggacagtagaaatatgaactatgtcatgctagggaagcccatgaacaatggactcatggagaagatggtggaggagagtgatgaggaagtgtgtctaagtagtctagagtgcctgaggaaccagtgctttgacctggccaggaaactcagcgagaccaacccacaggacaggagtcagccacccaacatgagtgtgcgccaacatgtccggcaagaggacgacttccctgggaggacgccagacaggagctactcggatatgatgaaccttatgcggctggaggagcagctcagtcccaggtctagaacgttctccagctgtgccaaggaggatgggtgtcatgagagggatgatgacaccacctcagtgaactcagacaggtctgaggaagtgtttgacatgaccaagggcaacctgactctgctagagaaagccattgccttggagacagagagagccaaggccatgcgggagaagatggccatggatgctgggagaagggataacctgagatcctatgaggaccagtctccaagacagctggctggggaagacagaaaatccaaatccagtgacagccatgtcaaaaagccatactatggtaaagatccctcaagaacagaaaagagagagagcaagtgtccaacccccgggtgtgatggaaccggccacgtaactgggctttacccgcatcaccgcagtctgtctggatgcccgcacaaagatagggtccctccagaaattcttgccatgcatgaaaatgttctcaagtgtcccactccaggctgcacagggcgagggcatgtgaatagcaacaggaactcgcacagaagcctctctggatgccccattgctgctgcagaaaaactggcaaaggcccaagagaaacaccagagctgtgatgtgtccaaatccaaccaggcctcagaccgagtcctcaggccaatgtgctttgtcaaacagcttgagattcctcagtatggctacagaaacaatgttcccacaaccacaccacgctccaacctggccaaggagcttgagaaatactccaagacttcgtttgagtacaacagttacgacaaccatacttatggcaaaagagccatagctcccaaggtgcaaaccagggacatatcccccaaaggatatgacgatgccaagcggtactgcaagaatgccagccccagcagcagcaccaccagcagctatgcacctagcagcagcagcaacctcagctgtggtggtggcagcagcgccagtagcacgtgtagcaagagcagctttgactacacacatgacatggaggccgcacacatggcagccacagccattctcaacctgtccacacgttgtcgtgaaatgccacagaacctgtccaccaagccacaggacctgtgtactgcccggaacccagacatggaggtggatgagaatggcaccctggacctgagcatgaacaagcagaggcctcgagacagctgctgcccagtcctgacacccctggaacccatgtctccgcagcagcaggccgtgatgagcagccgatgcttccagctgagcgagggggattgctgggacttgcctgtagactacaccaaaatgaagcctcggagggtagatgaggatgagcccaaagagattaccccagaagacttggacccattccaggaggctctggaagaaagacggtatccaggggaggtgaccatcccaagccccaaacccaagtaccctcagtgcaaggaaagcaaaaaggacttaataactctgtctggctgccccctggcggacaaaagcattcgaagtatgctggccaccagttcccaagagctcaagtgccccacccctggctgtgacggttctggacacatcactggcaattacgcttctcatcgaagcctttctgggtgcccgagagcaaagaagagtggcatccggatagcacagagcaaagaggacaaggaagaccaggagccaatcaggtgtccggtacctggctgtgacggtcagggacacatcactgggaagtatgcatcccaccgcagcgcctccgggtgtcccttggcagccaagaggcagaaagatgggtaccttaatggctcccagttctcctggaagtcggtcaagacggagggcatgtcctgccctacccccgggtgtgatgggtcaggacacgtcagtggcagcttcctcacacaccgcagcttgtcaggatgtccaagagccacatcagcaatgaagaaagcaaagctgtctggagaacagatgttgactatcaagcagcgagccagcaacggtatagaaaatgatgaagaaatcaagcagttagatgaagagatcaaggagcttaatgagtccaattcccagatggaggctgacatgatcaaactcagaactcagatcaccacaatggagagcaacctgaagacgattgaggaggagaacaaagtcattgaacagcagaatgagtcgctcttgcacgagttggccaacctgagccagtccctgatccacagcctcgccaacatccagctgcctcacatggatccaatcaatgaacaaaattttgatgcttacgtgactactttgacggaaatgtatacaaatcaagatcgttatcagagtccagaaaataaagccctactggaaaatataaagcaggctgtgagaggaattcaggtctga

SEQ ID NO: 23 - protein, 231 aa, synthetic construct
MGDMGDKKKRSCVGCGNHDYRVSDWHAACKCACNYDSCTCVRDGKTYCKRDYRYGKCAKCSGSKNDVMRARSKVYHCRCVACSRGDARDGCRADHDVVRASGAGDSHARMAASARARHVHKKTTRVRTVNKHTRTCYAANRDAMKVMTGSRVRVWNKRCKDKKRSMMKNDKTNGMTGTMVAASRHDGGANVVSYWKVSDASDDAVNSGGGSNSTGSVASMSSDTNSMVASA

SEQ ID NO: 24 - DNA, 1050 bp, synthetic construct
  source 1..1050: mol_type = other DNA
atgggagacatgggcgatccaccaaaaaaaaaacgtctgatttccctgtgtgttggttgcggcaatcaaattcacgaccagtatattctgagggtttctccggatttggagtggcatgcagcatgtttgaaatgtgcggagtgtaatcagtatttggacgaaagctgtacgtgctttgttagggatgggaaaacctactgtaaaagagattatatcaggttgtacgggatcaaatgcgccaagtgcagcataggcttcagcaagaacgacttcgtgatgcgtgcccgctctaaggtgtaccacatcgagtgtttccgctgtgtagcctgcagccgacagctcatcccgggagacgaattcgccctgcgggaggatgggcttttctgccgtgcagaccacgatgtggtggagagagccagcctgggagctggagaccctctcagtcccttgcatccagcgcggcctctgcaaatggcagccgaacccatctcggctaggcagccagctctgcggccgcacgtccacaagcagccggagaagaccacccgagtgcggactgtgctcaacgagaagcagctgcacaccttgcggacctgctatgccgccaaccctcggccagatgcgctcatgaaggagcaactagtggagatgacgggcctcagtcccagagtcatccgagtgtggtttcaaaacaagcggtgcaaggacaagaaacgcagcatcatgatgaagcagctccagcagcagcaacccaacgacaaaactaatatccaggggatgacaggaactcccatggtggctgctagtccggagagacatgatggtggtttacaggctaacccagtagaggtgcaaagttaccagccgccctggaaagtactgagtgacttcgccttgcaaagcgacatagatcagcctgcttttcagcaactggtcaatttttcagaaggaggaccaggctctaattctactggcagtgaagtagcatcgatgtcctcgcagctcccagatacacccaacagcatggtagccagtcctattgaggcatga

SEQ ID NO: 25 - protein, 178 aa, synthetic construct
MVKSTKVMGSASASATTMSSSADDRRGSARGRGAAGGVGSASGAGGCRGRGMHCKRRSRSRAVSRGAKTATVRKKTRRKANNRRNRMHNNAADARVTDAKTKTRAHNYWATTRADHCAGAGGGATAVSGAAGASGDSSSSWSCTNSASSSNSTSYSCTSASGSDVDYWKHRYAHARDC

SEQ ID NO: 26 - DNA, 792 bp, synthetic construct
  source 1..792: mol_type = other DNA
atgttcgtcaaatctgagactctggagttgaaggaggaagaggaggtactgatgctgctgggctcggcttccccggcctcggcgaccctgaccccgatgtcctccagcgcggacgaggaggaggacgaggagctgcgccggccgggctccgcgcgtgggcagcgtggagcggaagccgggcagggggtgcagggcagtccggcgtcgggtgccgggggttgccggccagggcggctgctgggcctgatgcacgagtgcaagcgtcgcccgtcgcgctcacgggccgtctcccgaggtgccaagacggcggagacggtgcagcgcatcaagaagacccgcaggctcaaggccaacaaccgcgagcgcaaccgcatgcacaacctaaacgccgcgctggacgcgctgcgcgaggtgctgcccaccttccccgaggatgccaagctcacgaagatcgagacgctgcgcttcgcccacaattacatctgggcgctcaccgagactctgcgcctggcggaccactgcgccggcgccggtggcctccagggggcgctcttcacggaggcggtgctcctgagcccgggagctgcgctcggcgccagcggggacagcccttctccaccttcctcctggagctgcaccaacagcccggcgtcatcctccaactccacgtccccatacagctgcactttatcgcccgctagccccgggtcagacgtggactactggcagcccccacctccggagaagcatcgttatgcgcctcacctgcccctcgccagggactgtatctag

SEQ ID NO: 27 - protein, 216 aa, synthetic construct
MTKSYSSGMGGSWTDCSSDHADKKDAMNADSRNGGDDDKKRRGKKKKMTKARRKRRMKANARRNRMHGNAADNRKVVCYSKTKSKTRAKNYWASRSGKSDVSVTCKGSTTNVAGCNRTNDMHTASASVHYSYSGSYGTMDSSHVHVKHAYSAASTDCTSSDGSSNGNSKHSAKNYATMHYAATAGSHGSSSGAAARCDNMSDSHSHHRVMSANAHD

SEQ ID NO: 28 - DNA, 1074 bp, synthetic construct
  source 1..1074: mol_type = other DNA
atgaccaaatcatacagcgagagcgggctgatgggcgagcctcagccccaaggtcccccaagctggacagatgagtgtctcagttctcaggacgaggaacacgaggcagacaagaaagaggacgagcttgaagccatgaatgcagaggaggactctctgagaaacgggggagaggaggaggaggaagatgaggatctagaggaagaggaggaagaagaagaggaggaggaggatcaaaagcccaagagacggggtcccaaaaagaaaaagatgaccaaggcgcgcctagaacgttttaaattaaggcgcatgaaggccaacgcccgcgagcggaaccgcatgcacgggctgaacgcggcgctggacaacctgcgcaaggtggtaccttgctactccaagacccagaaactgtctaaaatagagacactgcgcttggccaagaactacatctgggctctgtcagagatcctgcgctcaggcaaaagccctgatctggtctccttcgtacagacgctctgcaaaggtttgtcccagcccactaccaatttggtcgccggctgcctgcagctcaaccctcggactttcttgcctgagcagaacccggacatgcccccgcatctgccaaccgccagcgcttccttcccggtgcatccctactcctaccagtcccctggactgcccagcccgccctacggcaccatggacagctcccacgtcttccacgtcaagccgccgccacacgcctacagcgcagctctggagcccttctttgaaagccccctaactgactgcaccagcccttcctttgacggacccctcagcccgccgctcagcatcaatggcaacttctctttcaaacacgaaccatccgccgagtttgaaaaaaattatgcctttaccatgcactaccctgcagcgacgctggcagggccccaaagccacggatcaatcttctcttccggtgccgctgcccctcgctgcgagatccccatagacaacattatgtctttcgatagccattcgcatcatgagcgagtcatgagtgcccagcttaatgccatctttcacgattag

SEQ ID NO: 29 - DNA, 6952 bp, synthetic construct
  source 1..6952: mol_type = other DNA
cctgcaggcagctgcgcgctcgctcgctcactgaggccgcccgggcaaagcccgggcgtcgggcgacctttggtcgcccggcctcagtgagcgagcgagcgcgcagagagggagtggccaactccatcactaggggttccttctagacaactttgtatagaaaagttgtagttattaatagtaatcaattacggggtcattagttcatagcccatatatggagttccgcgttacataacttacggtaaatggcccgcctggctgaccgcccaacgacccccgcccattgacgtcaataatgacgtatgttcccatagtaacgccaatagggactttccattgacgtcaatgggtggagtatttacggtaaactgcccacttggcagtacatcaagtgtatcatatgccaagtacgccccctattgacgtcaatgacggtaaatggcccgcctggcattatgcccagtacatgaccttatgggactttcctacttggcagtacatctacgtattagtcatcgctattaccatggtgatgcggttttggcagtacatcaatgggcgtggatagcggtttgactcacggggatttccaagtctccaccccattgacgtcaatgggagtttgttttggcaccaaaatcaacgggactttccaaaatgtcgtaacaactccgccccattgacgcaaatgggcggtaggcgtgtacggtgggaggtctatataagcagagctggtttagtgaaccgtcagatccaagtttgtacaaaaaagcaggctgccaccatggaaaaatccaaaaatttccgcatcgacgccctgctggcggtggaccccccacgagccgcctctgcgcagagcgcgccgctggccttggtcacgtcgctcgccgccgccgcatctggcaccggaggtggcggcggcggcggcggggcgagcggcgggactagcggcagctgcagccccgcgtcctcggagccgccggctgcgcccgccgaccgcctgcgcgccgagagcccgtcgccgccgcgcctgctggccgcgcactgcgcgctgctgcccaagccgggcttcctgggcgcgggcggcggcggcggcggcacgggcggcgggcacggggggccccaccaccacgcgcatccgggcgcagcggccgctgccgccgccgccgccgccgccgccgccgctgggggcctggcgctggggctgcaccctgggggcgcgcagggcggcgcgggcctcccggcgcaggcggcgctctacggccacccggtctacggctactccgcggcggcggcggcggctgcgctggcgggccagcacccggcgctctcctactcgtacccgcaggtgcaaggcgcgcaccccgcgcaccccgccgaccccatcaagctgggcgccggcaccttccagctggaccagtggctgcgcgcgtccaccgcgggcatgatcctgcctaagatgcccgacttcaactcccaggcgcagtcgaacctcctggggaagtgccgccggccgcgcaccgccttcaccagccagcagctgctggagctggagcaccagttcaagctcaacaagtacctgtcgcggcccaagcgcttcgaggtggccacctcgctcatgctcaccgagacccaggtgaagatttggttccagaaccggcggatgaaatggaaacgcagcaaaaaggccaaagagcaggcggcgcaggaagcggagaaacagaagggcggcggcgggggcgcggggaagggcggcgcggaggagccgggagccgaggagctgctggggccgccagcgcccggagacaagggcagcggacgccgcctgcgggacttgagggacagtgaccccgaggaggacgaggacgaggacgacgaggaccatttcccctacagcaacggcgccagcgtccacgccgcctcctccgactgctcctcggaggacgactcgccgcccccgcggcccagccaccagcccgcgccccagggtagcggtgccactaacttctccctgttgaaacaagcaggggatgtcgaagagaatcctggtccaatggaagccagaggcgaactgggccctgccagagaatctgccggcggagatctgctgctggccctgctggctagaagggccgacctgagaagagaaatccccctgtgcgccggctgcgaccagcacatcctggaccggtttatcctgaaggccctggacagacactggcacagcaagtgcctgaagtgcagcgactgccacacccccctggccgagagatgctttagcagaggcgagagcgtgtactgcaaggacgacttcttcaagagattcggcaccaagtgcgccgcctgccagctgggaattcctcctacacaggtcgtgcggagagcccaggacttcgtgtaccatctgcactgcttcgcctgcgtcgtgtgcaagagacagctggccaccggcgacgagttctacctgatggaagatagccggctcgtgtgtaaagccgactacgagacagccaagcagagagaggccgaggccaccgccaaaagacccagaaccaccatcaccgccaagcagctggaaaccctgaagtccgcctacaacaccagccccaagcccgccagacatgtgcgggaacagctgagcagcgagacaggcctggacatgagagtggtgcaagtgtggttccagaacagacgggccaaagagaagcggctgaagaaggacgccggcaggcagagatggggccagtacttccggaacatgaagcggtccagaggcggcagcaagagcgacaaggacagcgtgcaggaaggccaggacagcgacgccgaggtgtccttcccagatgagcctagcctggccgaaatgggcccagccaatggcctgtatggcagcctgggagagccaacccaggctctgggcagaccttctggcgccctgggcaacttctctctggaacacggcggactggccggacccgagcagtatagagaactgaggcccggcagcccttacggcgtgccaccttctccagctgcccctcagtctctgccaggacctcagcctctgctgtccagcctggtgtaccccgatacaagcctgggcctggtgccatctggcgctccaggcggacctcctccaatgagagtgctggccggcaatggccctagcagcgatctgagcacaggcagctctggcggctaccccgattttcctgccagccctgcctcctggctggacgaagtggatcacgcccagttcggcagtggagagggcagaggaagtctgctaacatgcggtgacgtcgaggagaatcctggcccaatggcagcaaggcccaagctccactatcccaacggaagaggccggatggagtccgtgagatgggttttagctgccgccggagtcgagtttgatgaagaatttctggaaacaaaagaacagttgtacaagttgcaggatggtaaccacctgctgttccaacaagtgcccatggttgaaattgacgggatgaagttggtacagacccgaagcattctccactacatagcagacaagcacaatctctttggcaagaacctcaaggagagaaccctgattgacatgtacgtggaggggacactggatctgctggaactgcttatcatgcatcctttcttaaaaccagatgatcagcaaaaggaagtggttaacatggcccagaaggctataattagatactttcctgtgtttgaaaagattttaaggggtcacggacaaagctttcttgttggtaatcagctgagccttgcagatgtgattttactccaaaccattttagctctagaagagaaaattcctaatatcctgtctgcatttcctttcctccaggaatacacagtgaaactaagtaatatccctacaattaagagattccttgaacctggcagcaagaagaagcctccccctgatgaaatttatgtgagaaccgtctacaacatctttaggccataaacccagctttcttgtacaaagtgggaattcctagagctcgctgatcagcctcgactgtgccttctagttgccagccatctgttgtttgcccctcccccgtgccttccttgaccctggaaggtgccactcccactgtcctttcctaataaaatgaggaaattgcatcgcattgtctgagtaggtgtcattctattctggggggtggggtggggcaggacagcaagggggaggattgggaagagaatagcaggcatgctggggagggccgcaggaacccctagtgatggagttggccactccctctctgcgcgctcgctcgctcactgaggccgggcgaccaaaggtcgcccgacgcccgggctttgcccgggcggcctcagtgagcgagcgagcgcgcagctgcctgcaggggcgcctgatgcggtattttctccttacgcatctgtgcggtatttcacaccgcatacgtcaaagcaaccatagtacgcgccctgtagcggcgcattaagcgcggcgggtgtggtggttacgcgcagcgtgaccgctacacttgccagcgccttagcgcccgctcctttcgctttcttcccttcctttctcgccacgttcgccggctttccccgtcaagctctaaatcgggggctccctttagggttccgatttagtgctttacggcacctcgaccccaaaaaacttgatttgggtgatggttcacgtagtgggccatcgccctgatagacggtttttcgccctttgacgttggagtccacgttctttaatagtggactcttgttccaaactggaacaacactcaactctatctcgggctattcttttgatttataagggattttgccgatttcggtctattggttaaaaaatgagctgatttaacaaaaatttaacgcgaattttaacaaaatattaacgtttacaattttatggtgcactctcagtacaatctgctctgatgccgcatagttaagccagccccgacacccgccaacacccgctgacgcgccctgacgggcttgtctgctcccggcatccgcttacagacaagctgtgaccgtctccgggagctgcatgtgtcagaggttttcaccgtcatcaccgaaacgcgcgagacgaaagggcctcgtgatacgcctatttttataggttaatgtcatgataataatggtttcttagacgtcctggcccgtgtctcaaaatctctgatgttacattgcacaagataaaaatatatcatcatgaacaataaaactgtctgcttacataaacagtaatacaaggggtgttatgagccatattcaacgggaaacgtcgaggccgcgattaaattccaacatggatgctgatttatatgggtataaatgggctcgcgataatgtcgggcaatcaggtgcgacaatctatcgcttgtatgggaagcccgatgcgccagagttgtttctgaaacatggcaaaggtagcgttgccaatgatgttacagatgagatggtcagactaaactggctgacggaatttatgcctcttccgaccatcaagcattttatccgtactcctgatgatgcatggttactcaccactgcgatccccggaaaaacagcattccaggtattagaagaatatcctgattcaggtgaaaatattgttgatgcgctggcagtgttcctgcgccggttgcattcgattcctgtttgtaattgtccttttaacagcgatcgcgtatttcgtctcgctcaggcgcaatcacgaatgaataacggtttggttgatgcgagtgattttgatgacgagcgtaatggctggcctgttgaacaagtctggaaagaaatgcataaacttttgccattctcaccggattcagtcgtcactcatggtgatttctcacttgataaccttatttttgacgaggggaaattaataggttgtattgatgttggacgagtcggaatcgcagaccgataccaggatcttgccatcctatggaactgcctcggtgagttttctccttcattacagaaacggctttttcaaaaatatggtattgataatcctgatatgaataaattgcagtttcatttgatgctcgatgagtttttctaatcagaattggttaattggttgtaacactggcagagcattacgctgacttgacgggacggcgcaagctcatgaccaaaatcccttaacgtgagttacgcgtgaagatcctttttgataatctcatgaccaaaatcccttaacgtgagttttcgttccactgagcgtcagaccccgtagaaaagatcaaaggatcttcttgagatcctttttttctgcgcgtaatctgctgcttgcaaacaaaaaaaccaccgctaccagcggtggtttgtttgccggatcaagagctaccaactctttttccgaaggtaactggcttcagcagagcgcagataccaaatactgttcttctagtgtagccgtagttaggccaccacttcaagaactctgtagcaccgcctacatacctcgctctgctaatcctgttaccagtggctgctgccagtggcgataagtcgtgtcttaccgggttggactcaagacgatagttaccggataaggcgcagcggtcgggctgaacggggggttcgtgcacacagcccagcttggagcgaacgacctacaccgaactgagatacctacagcgtgagctatgagaaagcgccacgcttcccgaagggagaaaggcggacaggtatccggtaagcggcagggtcggaacaggagagcgcacgagggagcttccagggggaaacgcctggtatctttatagtcctgtcgggtttcgccacctctgacttgagcgtcgatttttgtgatgctcgtcaggggggcggagcctatggaaaaacgccagcaacgcggcctttttacggttcctggccttttgctggccttttgctcacatgt

SEQ ID NO: 30 - DNA, 20 bp, synthetic construct
  source 1..20: mol_type = other DNA
accttcctccatcctccctc

SEQ ID NO: 31 - DNA, 20 bp, synthetic construct
  source 1..20: mol_type = other DNA
tcctgctctgcgaattggtt

SEQ ID NO: 32 - DNA, 20 bp, synthetic construct
  source 1..20: mol_type = other DNA
tccagaaccgccgaatgaaa

SEQ ID NO: 33 - DNA, 20 bp, synthetic construct
  source 1..20: mol_type = other DNA
ccatcagctcctcttccgtc

SEQ ID NO: 34 - DNA, 20 bp, synthetic construct
  source 1..20: mol_type = other DNA
tcctcctgctcaacaacgac

SEQ ID NO: 35 - DNA, 20 bp, synthetic construct
  source 1..20: mol_type = other DNA
cggtccaaggccagaaagat

SEQ ID NO: 36 - DNA, 7059 bp, synthetic construct
  source 1..7059: mol_type = other DNA
cgccatgttgacattgattattgactagttattaatagtaatcaattacggggtcattagttcatagcccatatatggagttccgcgttacataacttacggtaaatggcccgcctggctgaccgcccaacgacccccgcccattgacgtcaataatgacgtatgttcccatagtaacgccaatagggactttccattgacgtcaatgggtggagtatttacggtaaactgcccacttggcagtacatcaagtgtatcatatgccaagtacgccccctattgacgtcaatgacggtaaatggcccgcctggcattatgcccagtacatgaccttatgggactttcctacttggcagtacatctacgtattagtcatcgctattaccatggtgatgcggttttggcagtacatcaatgggcgtggatagcggtttgactcacggggatttccaagtctccaccccattgacgtcaatgggagtttgttttggcaccaaaatcaacgggactttccaaaatgtcgtaacaactccgccccattgacgcaaatgggcggtaggcgtgtacggtgggaggtctatataagcagagctcgtttagtgaaccgtcagatcgcctggagacgccatccacgctgttttgacctccatagaagacaccgggaccgatccagcctcccctcgaagcttacatgtggtaccatggcagcaaggcccaagctccactatcccaacggaagaggccggatggagtccgtgagatgggttttagctgccgccggagtcgagtttgatgaagaatttctggaaacaaaagaacagttgtacaagttgcaggatggtaaccacctgctgttccaacaagtgcccatggttgaaattgacgggatgaagttggtacagacccgaagcattctccactacatagcagacaagcacaatctctttggcaagaacctcaaggagagaaccctgattgacatgtacgtggaggggacactggatctgctggaactgcttatcatgcatcctttcttaaaaccagatgatcagcaaaaggaagtggttaacatggcccagaaggctataattagatactttcctgtgtttgaaaagattttaaggggtcacggacaaagctttcttgttggtaatcagctgagccttgcagatgtgattttactccaaaccattttagctctagaagagaaaattcctaatatcctgtctgcatttcctttcctccaggaatacacagtgaaactaagtaatatccctacaattaagagattccttgaacctggcagcaagaagaagcctccccctgatgaaatttatgtgagaaccgtctacaacatctttaggccaggtagcggtgccactaacttctccctgttgaaacaagcaggggatgtcgaagagaatcctggtccaatggtgagcaagggcgaggagctgttcaccggggtggtgcccatcctggtcgagctggacggcgacgtaaacggccacaagttcagcgtgtccggcgagggcgagggcgatgccacctacggcaagctgaccctgaagttcatctgcaccaccggcaagctgcccgtgccctggcccaccctcgtgaccaccctgacctacggcgtgcagtgcttcagccgctaccccgaccacatgaagcagcacgacttcttcaagtccgccatgcccgaaggctacgtccaggagcgcaccatcttcttcaaggacgacggcaactacaagacccgcgccgaggtgaagttcgagggcgacaccctggtgaaccgcatcgagctgaagggcatcgacttcaaggaggacggcaacatcctggggcacaagctggagtacaactacaacagccacaacgtctatatcatggccgacaagcagaagaacggcatcaaggtgaacttcaagatccgccacaacatcgaggacggcagcgtgcagctcgccgaccactaccagcagaacacccccatcggcgacggccccgtgctgctgcccgacaaccactacctgagcacccagtccgccctgagcaaagaccccaacgagaagcgcgatcacatggtcctgctggagttcgtgaccgccgccgggatcactctcggcatggacgagctgtacaagtaaagcggccgctctagaggatccaagcttatcgataccgtcgacctcgagggcccagatctaattcaccccaccagtgcaggctgcctatcagaaagtggtggctggtgtggctaatgccctggcccacaagtatcactaagctcgctttcttgctgtccaatttctattaaaggttcctttgttccctaagtccaactactaaactgggggatattatgaagggccttgagcatctggattctgcctaataaaaaacatttattttcattgcaatgatgtatttaaattatttctgaatattttactaaaaagggaatgtgggaggtcagtgcatttaaaacataaagaaatgaagagctagttcaaaccttgggaaaatacactatatcttaaactccatgaaagaaggtgaggctgcaaacagctaatgcacattggcaacagcccctgatgcctatgccttattcatccctcagaaaaggattcaagtagaggcttgatttggaggttaaagttttgctatgctgtattttacattacttattgttttagctgtcctcatgaatgtcttttcactacccatttgcttatcctgcatctctcagccttgactccactcagttctcttgcttagagataccacctttcccctgaagtgttccttccatgttttacggcgagatggtttctcctcgcctggccactcagccttagttgtctctgttgtcttatagaggtctacttgaagaaggaaaaacagggggcatggtttgactgtcctgtgagcccttcttccctgcctcccccactcacagtgacccggaatccctcgacatctagagcatggctacgtagataagtagcatggcgggttaatcattaactacaaggaacccctagtgatggagttggccactccctctctgcgcgctcgctcgctcactgaggccgggcgaccaaaggtcgcccgacgcccgggctttgcccgggcggcctcagtgagcgagcgagcgcgcagctggcgtaatagcgaagaggcccgcaccgatcgcccttcccaacagttgcgcagcctgaatggcgaatggcgattccgttgcaatggctggcggtaatattgttctggatattaccagcaaggccgatagtttgagttcttctactcaggcaagtgatgttattactaatcaaagaagtattgcgacaacggttaatttgcgtgatggacagactcttttactcggtggcctcactgattataaaaacacttctcaggattctggcgtaccgttcctgtctaaaatccctttaatcggcctcctgtttagctcccgctctgattctaacgaggaaagcacgttatacgtgctcgtcaaagcaaccatagtacgcgccctgtagcggcgcattaagcgcggcgggtgtggtggttacgcgcagcgtgaccgctacacttgccagcgccctagcgcccgctcctttcgctttcttcccttcctttctcgccacgttcgccggctttccccgtcaagctctaaatcgggggctccctttagggttccgatttagtgctttacggcacctcgaccccaaaaaacttgattagggtgatggttcacgtagtgggccatcgccctgatagacggtttttcgccctttgacgttggagtccacgttctttaatagtggactcttgttccaaactggaacaacactcaaccctatctcggtctattcttttgatttataagggattttgccgatttcggcctattggttaaaaaatgagctgatttaacaaaaatttaacgcgaattttaacaaaatattaacgcttacaatttaaatatttgcttatacaatcttcctgtttttggggcttttctgattatcaaccggggtacatatgattgacatgctagttttacgattaccgttcatcgattctcttgtttgctccagactctcaggcaatgacctgatagcctttgtagagacctctcaaaaatagctaccctctccggcatgaatttatcagctagaacggttgaatatcatattgatggtgatttgactgtctccggcctttctcacccgtttgaatctttacctacacattactcaggcattgcatttaaaatatatgagggttctaaaaatttttatccttgcgttgaaataaaggcttctcccgcaaaagtattacagggtcataatgtttttggtacaaccgatttagctttatgctctgaggctttattgcttaattttgctaattctttgccttgcctgtatgatttattggatgttggaatcgcctgatgcggtattttctccttacgcatctgtgcggtatttcacaccgcatatggtgcactctcagtacaatctgctctgatgccgcatagttaagccagccccgacacccgccaacacccgctgacgcgccctgacgggcttgtctgctcccggcatccgcttacagacaagctgtgaccgtctccgggagctgcatgtgtcagaggttttcaccgtcatcaccgaaacgcgcgagacgaaagggcctcgtgatacgcctatttttataggttaatgtcatgataataatggtttcttagacgtcaggtggcacttttcggggaaatgtgcgcggaacccctatttgtttatttttctaaatacattcaaatatgtatccgctcatgagacaataaccctgataaatgcttcaataatattgaaaaaggaagagtatgagtattcaacatttccgtgtcgcccttattcccttttttgcggcattttgccttcctgtttttgctcacccagaaacgctggtgaaagtaaaagatgctgaagatcagttgggtgcacgagtgggttacatcgaactggatctcaacagcggtaagatccttgagagttttcgccccgaagaacgttttccaatgatgagcacttttaaagttctgctatgtggcgcggtattatcccgtattgacgccgggcaagagcaactcggtcgccgcatacactattctcagaatgacttggttgagtactcaccagtcacagaaaagcatcttacggatggcatgacagtaagagaattatgcagtgctgccataaccatgagtgataacactgcggccaacttacttctgacaacgatcggaggaccgaaggagctaaccgcttttttgcacaacatgggggatcatgtaactcgccttgatcgttgggaaccggagctgaatgaagccataccaaacgacgagcgtgacaccacgatgcctgtagcaatggcaacaacgttgcgcaaactattaactggcgaactacttactctagcttcccggcaacaattaatagactggatggaggcggataaagttgcaggaccacttctgcgctcggcccttccggctggctggtttattgctgataaatctggagccggtgagcgtgggtctcgcggtatcattgcagcactggggccagatggtaagccctcccgtatcgtagttatctacacgacggggagtcaggcaactatggatgaacgaaatagacagatcgctgagataggtgcctcactgattaagcattggtaactgtcagaccaagtttactcatatatactttagattgatttaaaacttcatttttaatttaaaaggatctaggtgaagatcctttttgataatctcatgaccaaaatcccttaacgtgagttttcgttccactgagcgtcagaccccgtagaaaagatcaaaggatcttcttgagatcctttttttctgcgcgtaatctgctgcttgcaaacaaaaaaaccaccgctaccagcggtggtttgtttgccggatcaagagctaccaactctttttccgaaggtaactggcttcagcagagcgcagataccaaatactgttcttctagtgtagccgtagttaggccaccacttcaagaactctgtagcaccgcctacatacctcgctctgctaatcctgttaccagtggctgctgccagtggcgataagtcgtgtcttaccgggttggactcaagacgatagttaccggataaggcgcagcggtcgggctgaacggggggttcgtgcacacagcccagcttggagcgaacgacctacaccgaactgagatacctacagcgtgagctatgagaaagcgccacgcttcccgaagggagaaaggcggacaggtatccggtaagcggcagggtcggaacaggagagcgcacgagggagcttccagggggaaacgcctggtatctttatagtcctgtcgggtttcgccacctctgacttgagcgtcgatttttgtgatgctcgtcaggggggcggagcctatggaaaaacgccagcaacgcggcctttttacggttcctggccttttgctggccttttgctcacatgttctttcctgcgttatcccctgattctgtggataaccgtattaccgcctttgagtgagctgataccgctcgccgcagccgaacgaccgagcgcagcgagtcagtgagcgaggaagcggaagagcgcccaatacgcaaaccgcctctccccgcgcgttggccgattcattaatgcagctgcgcgctcgctcgctcactgaggccgcccgggcaaagcccgggcgtcgggcgacctttggtcgcccggcctcagtgagcgagcgagcgcgcagagagggagtggccaactccatcactaggggttccttgtagttaatgattaacccgccatgctacttatctacgtagccatgctctagcggcctcggcctctgcataaataaaaaaaattagtcagccatgagcttggcccattgcatacgttgtatccatatcataatatgtacatttatattggctcatgtccaacattac